European Patent Specification EP 3 083 694 B1, published November 22, 2023. Title: CANINIZED MURINE ANTIBODIES TO HUMAN PD-1. Applicant: Intervet International BV Intervet Inc. Morsey, Mohamad Zhang, Yuanzheng Bartels-Morozov, Denise Erskine, Jason Tarpey, Ian Presta, Leonard G. The sequence listing filed with the application follows.

SEQUENCE LISTING (53 sequences)

SEQ ID NO: 1 - DNA, 795 bp, Canis familiaris
ctagactcccctgacaggccctggagcccgctcaccttctccccggcgcagctcacggtgcaggagggagagaacgccacgttcacctgcagcctggccgacatccccgacagcttcgtgctcaactggtaccgcctgagcccccgcaaccagacggacaagctggccgccttccaggaggaccgcatcgagccgggccgggacaggcgcttccgcgtcatgcggctgcccaacgggcgggacttccacatgagcatcgtcgctgcgcgcctcaacgacagcggcatctacctgtgcggggccatctacctgccccccaacacacagatcaacgagagtccccgcgcagagctctccgtgacggagagaaccctggagccccccacacagagccccagccccccacccagactcagcggccagttgcaggggctggtcatcggcgtcacgagcgtgctggtgggtgtcctgctactgctgctgctgacctgggtcctggccgctgtcttccccagggccacccgaggtgcctgtgtgtgcgggagcgaggacgagcctctgaaggagggccccgatgcagcgcccgtcttcaccctggactacggggagctggacttccagtggcgagagaagacgccggagcccccggcgccctgtgccccggagcagaccgagtatgccaccatcgtcttcccgggcaggccggcgtccccgggccgcagggcctcggccagcagcctgcagggagcccagcctccgagccccgaggacggacccggcctgtggcccctctga

SEQ ID NO: 2 - protein, 264 aa, Canis familiaris
LDSPDRPWSPLTFSPAQLTVQEGENATFTCSLADIPDSFVLNWYRLSPRNQTDKLAAFQEDRIEPGRDRRFRVMRLPNGRDFHMSIVAARLNDSGIYLCGAIYLPPNTQINESPRAELSVTERTLEPPTQSPSPPPRLSGQLQGLVIGVTSVLVGVLLLLLLTWVLAAVFPRATRGACVCGSEDEPLKEGPDAAPVFTLDYGELDFQWREKTPEPPAPCAPEQTEYATIVFPGRPASPGRRASASSLQGAQPPSPEDGPGLWPL

SEQ ID NO: 3 - DNA, 438 bp, Artificial Sequence
  codon optimized
ctggattcccccgacagaccctggagccctctcaccttctcccctgcccagctgaccgtccaggaaggcgagaatgccaccttcacctgcagcctcgccgacatccccgacagcttcgtgctgaactggtacagactgagccccaggaaccagaccgacaagctggccgctttccaggaggacaggatcgaacccggcagggacaggaggtttagggtcatgaggctgcccaacggcagggacttccacatgtccatcgtggccgccagactgaacgactccggcatctacctgtgcggcgctatctacctgccccccaacacccagatcaacgagagccccagggccgaactgagcgtgacagagagaaccctggaacctcccacccagagcccttcccctcctcctagactgagcggacagctgcagggcctggtg

SEQ ID NO: 4 - protein, 146 aa, Canis familiaris
LDSPDRPWSPLTFSPAQLTVQEGENATFTCSLADIPDSFVLNWYRLSPRNQTDKLAAFQEDRIEPGRDRRFRVMRLPNGRDFHMSIVAARLNDSGIYLCGAIYLPPNTQINESPRAELSVTERTLEPPTQSPSPPPRLSGQLQGLV

SEQ ID NO: 5 - DNA, 1128 bp, Artificial Sequence
  codon optimized
ctggattcccccgacagaccctggagccctctcaccttctcccctgcccagctgaccgtccaggaaggcgagaatgccaccttcacctgcagcctcgccgacatccccgacagcttcgtgctgaactggtacagactgagccccaggaaccagaccgacaagctggccgctttccaggaggacaggatcgaacccggcagggacaggaggtttagggtcatgaggctgcccaacggcagggacttccacatgtccatcgtggccgccagactgaacgactccggcatctacctgtgcggcgctatctacctgccccccaacacccagatcaacgagagccccagggccgaactgagcgtgacagagagaaccctggaacctcccacccagagcccttcccctcctcctagactgagcggacagctgcagggcctggtgggtaccgacaaaactcacacatgcccaccgtgcccagcacctgaactcctggggggaccgtcagtcttcctcttccccccaaaacccaaggacaccctcatgatctcccggacccctgaggtcacatgcgtggtggtggacgtgagccacgaagaccctgaggtcaagttcaactggtacgtggacggcgtggaggtgcataatgccaagacaaagccgcgggaggagcagtacaacagcacgtaccgtgtggtcagcgtcctcaccgtcctgcaccaggactggctgaatggcaaggagtacaagtgcaaggtctccaacaaagccctcccagcccccatcgagaaaaccatctccaaagccaaagggcagccccgagaaccacaggtgtacaccctgcccccatcccgggatgagctgaccaagaaccaggtcagcctgacctgcctggtcaaaggcttctatcccagcgacatcgccgtggagtgggagagcaatgggcagccggagaacaactacaagaccacgcctcccgtgctggactccgacggctccttcttcctctacagcaagctcaccgtggacaagagcaggtggcagcaggggaacgtcttctcatgctccgtgatgcatgaggctctgcacaaccactacacgcagaagagcctctccctgtctccgggtaaatga

SEQ ID NO: 6 - protein, 375 aa, Artificial Sequence
  canine and human
LDSPDRPWSPLTFSPAQLTVQEGENATFTCSLADIPDSFVLNWYRLSPRNQTDKLAAFQEDRIEPGRDRRFRVMRLPNGRDFHMSIVAARLNDSGIYLCGAIYLPPNTQINESPRAELSVTERTLEPPTQSPSPPPRLSGQLQGLVGTDKTHTCPPCPAPELLGGPSVFLFPPKPKDTLMISRTPEVTCVVVDVSHEDPEVKFNWYVDGVEVHNAKTKPREEQYNSTYRVVSVLTVLHQDWLNGKEYKCKVSNKALPAPIEKTISKAKGQPREPQVYTLPPSRDELTKNQVSLTCLVKGFYPSDIAVEWESNGQPENNYKTTPPVLDSDGSFFLYSKLTVDKSRWQQGNVFSCSVMHEALHNHYTQKSLSLSPGK

SEQ ID NO: 7 - DNA, 816 bp, Canis familiaris
tttacgatcacagtttctaaggacctgtatgtggtagagtatggtggcaatgtgacaatggaatgcaaattcccggtggaaaaacagttaaacttgtttgcactaatcgtctactgggaaatggaggataaaaaaattatacaatttgtgaatggaaaggaagacctgaaagttcagcacagcagctacagccagagggctcagctattgaaggaccagctcttcttggggaaggctgcgcttcagatcacagatgtgagattgcaggatgcaggggtttactgctgcttgatcggctatggcggtgctgactacaagcggattactttgaaagttcatgccccgtaccgcaacatcagccaaagaatttctgtggatcctgtcacctctgaacatgaactaatgtgtcaggctgagggttaccctgaggctgaagtcatctggacaagcagtgaccaccgagtcctgagtggcaaaaccaccatcactaattccaatagggaagagaagcttttcaatgtgaccagcacgctgaacatcaatgcaacagctaatgagattttctactgcacttttcaaagatcaggtcctgaggaaaacaatactgccgagttggtcatcccagaacgactgcccgttccagcaagtgagaggactcatttcatgattctgggacctttcctgttgcttcttggtgtagtcctggcagtcactttctgtctaaaaaaacatgggagaatgatggatgtggaaaaatgttgcacccgagataggaactcaaagaaacgaaatgatatacaatttgaagagacataa

SEQ ID NO: 8 - protein, 271 aa, Canis familiaris
FTITVSKDLYVVEYGGNVTMECKFPVEKQLNLFALIVYWEMEDKKIIQFVNGKEDLKVQHSSYSQRAQLLKDQLFLGKAALQITDVRLQDAGVYCCLIGYGGADYKRITLKVHAPYRNISQRISVDPVTSEHELMCQAEGYPEAEVIWTSSDHRVLSGKTTITNSNREEKLFNVTSTLNINATANEIFYCTFQRSGPEENNTAELVIPERLPVPASERTHFMILGPFLLLLGVVLAVTFCLKKHGRMMDVEKCCTRDRNSKKRNDIQFEET

SEQ ID NO: 9 - DNA, 660 bp, Artificial Sequence
  codon optimized
tttaccatcaccgtgtccaaggacctgtacgtggtcgagtacggcggcaatgtgaccatggagtgcaagttccccgtggagaagcagctgaacctgttcgccctcatcgtgtactgggagatggaggacaagaagatcatccagttcgtgaacggcaaggaggacctgaaggtgcagcactccagctactcccagagagcccagctgctgaaggaccagctgttcctgggcaaggccgccctgcagatcaccgacgtgagactgcaggacgccggcgtgtattgctgcctgatcggctacggaggcgccgactacaagaggatcaccctgaaggtgcatgcaccctacaggaacatcagccagaggatcagcgtcgatcccgtgaccagcgagcacgagctgatgtgccaagccgagggctatcccgaggccgaagtgatctggaccagcagcgaccacagggtcctgagcggcaagaccaccatcaccaacagcaacagggaggagaagctgttcaacgtgaccagcaccctcaacatcaacgccaccgccaacgagatcttctactgcaccttccagaggagcggccccgaagagaacaacaccgccgagctggtgatccccgagagactgcctgtgcctgccagcgagaggacccac

SEQ ID NO: 10 - protein, 220 aa, Canis familiaris
FTITVSKDLYVVEYGGNVTMECKFPVEKQLNLFALIVYWEMEDKKIIQFVNGKEDLKVQHSSYSQRAQLLKDQLFLGKAALQITDVRLQDAGVYCCLIGYGGADYKRITLKVHAPYRNISQRISVDPVTSEHELMCQAEGYPEAEVIWTSSDHRVLSGKTTITNSNREEKLFNVTSTLNINATANEIFYCTFQRSGPEENNTAELVIPERLPVPASERTH

SEQ ID NO: 11 - DNA, 1350 bp, Artificial Sequence
  codon optimized
tttaccatcaccgtgtccaaggacctgtacgtggtcgagtacggcggcaatgtgaccatggagtgcaagttccccgtggagaagcagctgaacctgttcgccctcatcgtgtactgggagatggaggacaagaagatcatccagttcgtgaacggcaaggaggacctgaaggtgcagcactccagctactcccagagagcccagctgctgaaggaccagctgttcctgggcaaggccgccctgcagatcaccgacgtgagactgcaggacgccggcgtgtattgctgcctgatcggctacggaggcgccgactacaagaggatcaccctgaaggtgcatgcaccctacaggaacatcagccagaggatcagcgtcgatcccgtgaccagcgagcacgagctgatgtgccaagccgagggctatcccgaggccgaagtgatctggaccagcagcgaccacagggtcctgagcggcaagaccaccatcaccaacagcaacagggaggagaagctgttcaacgtgaccagcaccctcaacatcaacgccaccgccaacgagatcttctactgcaccttccagaggagcggccccgaagagaacaacaccgccgagctggtgatccccgagagactgcctgtgcctgccagcgagaggacccacggtaccgacaaaactcacacatgcccaccgtgcccagcacctgaactcctggggggaccgtcagtcttcctcttccccccaaaacccaaggacaccctcatgatctcccggacccctgaggtcacatgcgtggtggtggacgtgagccacgaagaccctgaggtcaagttcaactggtacgtggacggcgtggaggtgcataatgccaagacaaagccgcgggaggagcagtacaacagcacgtaccgtgtggtcagcgtcctcaccgtcctgcaccaggactggctgaatggcaaggagtacaagtgcaaggtctccaacaaagccctcccagcccccatcgagaaaaccatctccaaagccaaagggcagccccgagaaccacaggtgtacaccctgcccccatcccgggatgagctgaccaagaaccaggtcagcctgacctgcctggtcaaaggcttctatcccagcgacatcgccgtggagtgggagagcaatgggcagccggagaacaactacaagaccacgcctcccgtgctggactccgacggctccttcttcctctacagcaagctcaccgtggacaagagcaggtggcagcaggggaacgtcttctcatgctccgtgatgcatgaggctctgcacaaccactacacgcagaagagcctctccctgtctccgggtaaatga

SEQ ID NO: 12 - protein, 449 aa, Canis familiaris
FTITVSKDLYVVEYGGNVTMECKFPVEKQLNLFALIVYWEMEDKKIIQFVNGKEDLKVQHSSYSQRAQLLKDQLFLGKAALQITDVRLQDAGVYCCLIGYGGADYKRITLKVHAPYRNISQRISVDPVTSEHELMCQAEGYPEAEVIWTSSDHRVLSGKTTITNSNREEKLFNVTSTLNINATANEIFYCTFQRSGPEENNTAELVIPERLPVPASERTHGTDKTHTCPPCPAPELLGGPSVFLFPPKPKDTLMISRTPEVTCVVVDVSHEDPEVKFNWYVDGVEVHNAKTKPREEQYNSTYRVVSVLTVLHQDWLNGKEYKCKVSNKALPAPIEKTISKAKGQPREPQVYTLPPSRDELTKNQVSLTCLVKGFYPSDIAVEWESNGQPENNYKTTPPVLDSDGSFFLYSKLTVDKSRWQQGNVFSCSVMHEALHNHYTQKSLSLSPGK

SEQ ID NO: 13 - DNA, 15 bp, Mus musculus
agttattatctgtac

SEQ ID NO: 14 - protein, 5 aa, Mus musculus
SYYLY

SEQ ID NO: 15 - DNA, 48 bp, Mus musculus
ggggttaatcctagtaatggtggtactaacttcagtgagaagttcaag

SEQ ID NO: 16 - protein, 16 aa, Mus musculus
GVNPSNGGTNFSEKFK

SEQ ID NO: 17 - DNA, 33 bp, Mus musculus
agggattctaactacgacgggggctttgactac

SEQ ID NO: 18 - protein, 11 aa, Mus musculus
RDSNYDGGFDY

SEQ ID NO: 19 - DNA, 45 bp, Mus musculus
agggccagcaaaagtgtcagtacatctggctttagttatttgcac

SEQ ID NO: 20 - protein, 15 aa, Mus musculus
RASKSVSTSGFSYLH

SEQ ID NO: 21 - DNA, 21 bp, Mus musculus
cttgcatccaacctagagtct

SEQ ID NO: 22 - protein, 7 aa, Mus musculus
LASNLES

SEQ ID NO: 23 - DNA, 27 bp, Mus musculus
cagcacagttgggagcttccgctcacg

SEQ ID NO: 24 - protein, 9 aa, Mus musculus
QHSWELPLT

SEQ ID NO: 25 - DNA, 1353 bp, Artificial Sequence
  caninized mouse antibody
gaggtgcagctggtgcagtccggcggcgatctggtgaagcctggaggcagcgtgagactgagctgcgtggccagcggctacaccttcaccagctactacctgtactgggtgaggcaggctcctggcaaaggactgcagtggatcggcggcgtgaatcctagcaacggcggcaccaacttcagcgagaagttcaagagcagggccaccctgagcgtggacaaggccaagaacaccgcctacatgcagctgaactccctgagggccgaggacaccgccgtgtactactgcaccaggagggacagcaactacgacggcggcttcgactactggggacagggaaccctgctgaccgtgtccagcgcttccacaacggctccgtcggtgtttcccctggcacctagctgcgggtcgacctcgggtagcacagtggcgctggcgtgtttggtgtcgggatactttcccgagccggtaacggtgtcatggaactcagggtcacttacatcaggagtccatacttttccgtccgtgctgcagtcaagcggcttgcattcactgtcctcgatggtgacggtgccttcgtcgaggtggcccagcgaaacgttcacttgtaacgtagtacacccggcctccaacacgaaagtcgataaaccggtattcaatgagtgcagatgtacagacacccctccctgtccggtacccgaaccccttggagggccgagcgtcctcatcttccctcccaagccaaaagacatcttgcgcattacgaggacaccagaagtcacgtgcgtagtgcttgatctcggtagagaagatcccgaggtccagatctcgtggtttgtggatggaaaggaggtccacaccgcaaagactcagtcgcgcgagcagcagttcaatggcacgtatcgggtcgtgagcgtgcttcctatcgagcatcaggactggctcaccgggaaggagttcaaatgccgggtcaatcatatcgacctcccgtcaccaatcgagcggaccatctcgaaggctagaggaagggcgcacaaaccttcggtctatgtgcttcccccatcgcccaaagagctttcctcgtcggatacggtgtccattacatgcttgattaaggacttctatcctcctgatattgatgtggaatggcaatcaaacggacagcaggagccggaacgcaagcaccgaatgaccccaccgcaattggacgaagatggtagctactttctctactcaaagctctcagtcgacaaatcccgatggcagcagggagatcccttcacttgcgccgtgatgcacgagacactccaaaatcattacacggacctttcgttgagccactcgcccggaaag

SEQ ID NO: 26 - protein, 451 aa, Artificial Sequence
  caninized mouse antibody
EVQLVQSGGDLVKPGGSVRLSCVASGYTFTSYYLYWVRQAPGKGLQWIGGVNPSNGGTNFSEKFKSRATLSVDKAKNTAYMQLNSLRAEDTAVYYCTRRDSNYDGGFDYWGQGTLLTVSSASTTAPSVFPLAPSCGSTSGSTVALACLVSGYFPEPVTVSWNSGSLTSGVHTFPSVLQSSGLHSLSSMVTVPSSRWPSETFTCNVVHPASNTKVDKPVFNECRCTDTPPCPVPEPLGGPSVLIFPPKPKDILRITRTPEVTCVVLDLGREDPEVQISWFVDGKEVHTAKTQSREQQFNGTYRVVSVLPIEHQDWLTGKEFKCRVNHIDLPSPIERTISKARGRAHKPSVYVLPPSPKELSSSDTVSITCLIKDFYPPDIDVEWQSNGQQEPERKHRMTPPQLDEDGSYFLYSKLSVDKSRWQQGDPFTCAVMHETLQNHYTDLSLSHSPGK

SEQ ID NO: 27 - DNA, 1368 bp, Artificial Sequence
  caninized mouse antibody
gaggtgcagctggtgcagtccggcggcgatctggtgaagcctggaggcagcgtgagactgagctgcgtggccagcggctacaccttcaccagctactacctgtactgggtgaggcaggctcctggcaaaggactgcagtggatcggcggcgtgaatcctagcaacggcggcaccaacttcagcgagaagttcaagagcagggccaccctgagcgtggacaaggccaagaacaccgcctacatgcagctgaactccctgagggccgaggacaccgccgtgtactactgcaccaggagggacagcaactacgacggcggcttcgactactggggacagggaaccctgctgaccgtgtccagcgcttccacaaccgcgccatcagtctttccgttggccccatcatgcgggtcgacgagcggatcgactgtggccctggcgtgcttggtgtcgggatactttcccgaacccgtcacggtcagctggaactccggatcgcttacgagcggtgtgcatacgttcccctcggtcttgcaatcatcagggctctactcgctgtcgagcatggtaacggtgccctcatcgaggtggccctccgaaacgttcacatgtaacgtagcacatccagcctccaaaaccaaggtggataaacccgtgccgaaaagagagaatgggcgggtgcctcgaccccctgattgccccaagtgtccggctccggaaatgctcggtggaccctcagtgtttatcttccctccgaagcccaaggacactctgctgatcgcgcgcactccagaagtaacatgtgtagtggtggaccttgatcccgaggaccccgaagtccagatctcctggtttgtagatgggaaacagatgcagaccgcaaaaactcaacccagagaggagcagttcaacggaacataccgagtggtatccgtccttccgattggccaccaggactggttgaaagggaagcagtttacgtgtaaagtcaacaataaggcgttgcctagccctattgagcggacgatttcgaaagctaggggacaggcccaccagccatcggtctatgtccttccgccttcccgcgaggagctctcgaagaatacagtgagccttacatgcctcattaaggatttcttcccgcctgatatcgacgtagagtggcaatcaaacggtcaacaggagccggaatccaagtatagaaccactccgccccagcttgacgaggacggatcatactttttgtattcaaaactgtcggtggataagagccggtggcagagaggtgacaccttcatctgtgcggtgatgcacgaagcactccataatcactacacccaagagagcctctcgcattcccccggaaagtga

SEQ ID NO: 28 - protein, 455 aa, Artificial Sequence
  caninized mouse antibody
EVQLVQSGGDLVKPGGSVRLSCVASGYTFTSYYLYWVRQAPGKGLQWIGGVNPSNGGTNFSEKFKSRATLSVDKAKNTAYMQLNSLRAEDTAVYYCTRRDSNYDGGFDYWGQGTLLTVSSASTTAPSVFPLAPSCGSTSGSTVALACLVSGYFPEPVTVSWNSGSLTSGVHTFPSVLQSSGLYSLSSMVTVPSSRWPSETFTCNVAHPASKTKVDKPVPKRENGRVPRPPDCPKCPAPEMLGGPSVFIFPPKPKDTLLIARTPEVTCVVVDLDPEDPEVQISWFVDGKQMQTAKTQPREEQFNGTYRVVSVLPIGHQDWLKGKQFTCKVNNKALPSPIERTISKARGQAHQPSVYVLPPSREELSKNTVSLTCLIKDFFPPDIDVEWQSNGQQEPESKYRTTPPQLDEDGSYFLYSKLSVDKSRWQRGDTFICAVMHEALHNHYTQESLSHSPGK

SEQ ID NO: 29 - DNA, 1353 bp, Artificial Sequence
  caninized mouse antibody
gaggtgcagctggtgcagtccggcggcgatctggtgaagcctggaggcagcgtgagactgagctgcgtggccagcggctacaccttcaccagctactacctgtactgggtgaggcaggctcctggcaaaggactgcagtggatcggcggcgtgaatcctagcaacggcggcaccaacttcagcgagaagttcaagagcagggccaccctgagcgtggacaaggccaagaacaccgcctacatgcagctgaactccctgagggccgaggacaccgccgtgtactactgcaccaggagggacagcaactacgacggcggcttcgactactggggacagggaaccctgctgaccgtgtccagcgcttcaaccacagcgccgagcgtgttccctctggcgccgtcgtgcggttccacctcgggatcaacagtggccctcgcctgtctcgtgagcggatactttccggagcctgtcacggtgtcgtggaatagcggatcactcacgtcgggcgtgcatacttttccatccgtcttgcaatcgagcggattgtactcactctcctcaaccgtcactgtcccctcgtcgcgctggccctcggagacttttacgtgcaatgtagtccatccggcgagcaacacgaaggtcgacaagcccgtacccaaggaatcaacatgcaagtgcatctcgccctgtcccgtccccgaatcccttggtggcccctcagtgtttatcttccctccgaagcctaaagacatcttgagaatcacaagaacaccggaaatcacgtgtgtggtccttgacttgggacgcgaggaccctgaggtacaaatctcgtggtttgtggacgggaaagaggtgcacacagcaaagacacaaccacgcgagcagcagtttaactcaacgtacagggtagtatccgtacttcccattgaacaccaggattggctcaccggtaaagaattcaaatgccgagtgaatcacatcgggcttcctagcccaattgagcggacgatttccaaagctaggggtcaggcccaccagccgagcgtatacgtgttgccgccctccccgaaggagctgtcatcgtcagatacggtaacgttgacgtgtctgatcaaagatttctttcctcccgaaattgatgtggaatggcaaagcaatgggcagcccgagcccgagtcaaagtaccatactactgcaccacagctggacgaagatggatcgtatttcctctactcgaaactgtccgtggataagtcccggtggcagcaaggggacaccttcacttgcgcggtcatgcacgaggcacttcagaaccactatacggacttgagcctctcgcattcgccagggaag

SEQ ID NO: 30 - protein, 451 aa, Artificial Sequence
  caninized mouse antibody
EVQLVQSGGDLVKPGGSVRLSCVASGYTFTSYYLYWVRQAPGKGLQWIGGVNPSNGGTNFSEKFKSRATLSVDKAKNTAYMQLNSLRAEDTAVYYCTRRDSNYDGGFDYWGQGTLLTVSSASTTAPSVFPLAPSCGSTSGSTVALACLVSGYFPEPVTVSWNSGSLTSGVHTFPSVLQSSGLYSLSSTVTVPSSRWPSETFTCNVVHPASNTKVDKPVPKESTCKCISPCPVPESLGGPSVFIFPPKPKDILRITRTPEITCVVLDLGREDPEVQISWFVDGKEVHTAKTQPREQQFNSTYRVVSVLPIEHQDWLTGKEFKCRVNHIGLPSPIERTISKARGQAHQPSVYVLPPSPKELSSSDTVTLTCLIKDFFPPEIDVEWQSNGQPEPESKYHTTAPQLDEDGSYFLYSKLSVDKSRWQQGDTFTCAVMHEALQNHYTDLSLSHSPGK

SEQ ID NO: 31 - DNA, 666 bp, Artificial Sequence
  caninized mouse antibody
gatatcgtcctgacccagacccctctgagcctgtccgtgagccctggagaacccgccagcatcagctgcagggcctccaagagcgtgagcaccagcggcttcagctacctgcactggtacaggcagaagcccggacagagccctcagctgctgatcttcctggccagcaacctggagagcggcgtgcctgacaggtttagcggaagcggcagcggcaccgacttcacactgaggatctccagggtggaagccgacgacgccggagtgtactactgccagcacagctgggaactgcccctgaccttcggccagggcaccaaggtggagatcaagaggaacgacgctcagccagccgtgtacctcttccagccttcgccggaccagcttcatacggggtcagcgtcggtggtgtgcctgttgaactcgttttaccccaaggacattaacgtgaagtggaaggtagacggggtaattcaagacactggcattcaagagtccgtcacggaacaagactcaaaagactcaacgtattcactgtcgtcaaccttgacgatgtcaagcaccgagtatcttagccatgagctgtattcgtgcgagatcacccacaagtccctcccctccactcttatcaaatcctttcagcggtcggaatgtcagcgggtcgat

SEQ ID NO: 32 - protein, 222 aa, Artificial Sequence
  caninized mouse antibody
DIVLTQTPLSLSVSPGEPASISCRASKSVSTSGFSYLHWYRQKPGQSPQLLIFLASNLESGVPDRFSGSGSGTDFTLRISRVEADDAGVYYCQHSWELPLTFGQGTKVEIKRNDAQPAVYLFQPSPDQLHTGSASVVCLLNSFYPKDINVKWKVDGVIQDTGIQESVTEQDSKDSTYSLSSTLTMSSTEYLSHELYSCEITHKSLPSTLIKSFQRSECQRVD

SEQ ID NO: 33 - DNA, 666 bp, Artificial Sequence
  caninized mouse antibody
gatatcgtcctgacccagacccctcctagcctgtccgtgagccctggagaacccgccagcatcagctgcagggcctccaagagcgtgagcaccagcggcttcagctacctgcactggtacaggcagaagcccggacagcctcctcagctgctgatcttcctggccagcaacctggagagcggcgtgcctgacaggtttagcggaagcggcagcggcaccgacttcacactgaggatctccagggtggaagccgacgacgccggagtgtactactgccagcacagctgggaactgcccctgaccttcggccagggcaccaaggtggagatcaagaggaacgacgctcagccagccgtgtacctcttccagccttcgccggaccagcttcatacggggtcagcgtcggtggtgtgcctgttgaactcgttttaccccaaggacattaacgtgaagtggaaggtagacggggtaattcaagacactggcattcaagagtccgtcacggaacaagactcaaaagactcaacgtattcactgtcgtcaaccttgacgatgtcaagcaccgagtatcttagccatgagctgtattcgtgcgagatcacccacaagtccctcccctccactcttatcaaatcctttcagcggtcggaatgtcagcgggtcgat

SEQ ID NO: 34 - protein, 222 aa, Artificial Sequence
  caninized mouse antibody
DIVLTQTPPSLSVSPGEPASISCRASKSVSTSGFSYLHWYRQKPGQPPQLLIFLASNLESGVPDRFSGSGSGTDFTLRISRVEADDAGVYYCQHSWELPLTFGQGTKVEIKRNDAQPAVYLFQPSPDQLHTGSASVVCLLNSFYPKDINVKWKVDGVIQDTGIQESVTEQDSKDSTYSLSSTLTMSSTEYLSHELYSCEITHKSLPSTLIKSFQRSECQRVD

SEQ ID NO: 35 - DNA, 867 bp, Canis familiaris
atggggagccggcgggggccctggccgctcgtctgggccgtgctgcagctgggctggtggccaggatggctcctagactcccctgacaggccctggagcccgctcaccttctccccggcgcagctcacggtgcaggagggagagaacgccacgttcacctgcagcctggccgacatccccgacagcttcgtgctcaactggtaccgcctgagcccccgcaaccagacggacaagctggccgccttccaggaggaccgcatcgagccgggccgggacaggcgcttccgcgtcatgcggctgcccaacgggcgggacttccacatgagcatcgtcgctgcgcgcctcaacgacagcggcatctacctgtgcggggccatctacctgccccccaacacacagatcaacgagagtccccgcgcagagctctccgtgacggagagaaccctggagccccccacacagagccccagccccccacccagactcagcggccagttgcaggggctggtcatcggcgtcacgagcgtgctggtgggtgtcctgctactgctgctgctgacctgggtcctggccgctgtcttccccagggccacccgaggtgcctgtgtgtgcgggagcgaggacgagcctctgaaggagggccccgatgcagcgcccgtcttcaccctggactacggggagctggacttccagtggcgagagaagacgccggagcccccggcgccctgtgccccggagcagaccgagtatgccaccatcgtcttcccgggcaggccggcgtccccgggccgcagggcctcggccagcagcctgcagggagcccagcctccgagccccgaggacggacccggcctgtggcccctctga

SEQ ID NO: 36 - protein, 288 aa, Canis familiaris
MGSRRGPWPLVWAVLQLGWWPGWLLDSPDRPWSPLTFSPAQLTVQEGENATFTCSLADIPDSFVLNWYRLSPRNQTDKLAAFQEDRIEPGRDRRFRVMRLPNGRDFHMSIVAARLNDSGIYLCGAIYLPPNTQINESPRAELSVTERTLEPPTQSPSPPPRLSGQLQGLVIGVTSVLVGVLLLLLLTWVLAAVFPRATRGACVCGSEDEPLKEGPDAAPVFTLDYGELDFQWREKTPEPPAPCAPEQTEYATIVFPGRPASPGRRASASSLQGAQPPSPEDGPGLWPL

SEQ ID NO: 37 - DNA, 870 bp, Canis familiaris
atgagaatgtttagtgtctttacattcatggcctactgccatttgctaaaagcatttacgatcacagtttctaaggacctgtatgtggtagagtatggtggcaatgtgacaatggaatgcaaattcccggtggaaaaacagttaaacttgtttgcactaatcgtctactgggaaatggaggataaaaaaattatacaatttgtgaatggaaaggaagacctgaaagttcagcacagcagctacagccagagggctcagctattgaaggaccagctcttcttggggaaggctgcgcttcagatcacagatgtgagattgcaggatgcaggggtttactgctgcttgatcggctatggcggtgctgactacaagcggattactttgaaagttcatgccccgtaccgcaacatcagccaaagaatttctgtggatcctgtcacctctgaacatgaactaatgtgtcaggctgagggttaccctgaggctgaagtcatctggacaagcagtgaccaccgagtcctgagtggcaaaaccaccatcactaattccaatagggaagagaagcttttcaatgtgaccagcacgctgaacatcaatgcaacagctaatgagattttctactgcacttttcaaagatcaggtcctgaggaaaacaatactgccgagttggtcatcccagaacgactgcccgttccagcaagtgagaggactcatttcatgattctgggacctttcctgttgcttcttggtgtagtcctggcagtcactttctgtctaaaaaaacatgggagaatgatggatgtggaaaaatgttgcacccgagataggaactcaaagaaacgaaatgatatacaatttgaagagacataa

SEQ ID NO: 38 - protein, 289 aa, Canis familiaris
MRMFSVFTFMAYCHLLKAFTITVSKDLYVVEYGGNVTMECKFPVEKQLNLFALIVYWEMEDKKIIQFVNGKEDLKVQHSSYSQRAQLLKDQLFLGKAALQITDVRLQDAGVYCCLIGYGGADYKRITLKVHAPYRNISQRISVDPVTSEHELMCQAEGYPEAEVIWTSSDHRVLSGKTTITNSNREEKLFNVTSTLNINATANEIFYCTFQRSGPEENNTAELVIPERLPVPASERTHFMILGPFLLLLGVVLAVTFCLKKHGRMMDVEKCCTRDRNSKKRNDIQFEET

SEQ ID NO: 39 - DNA, 1410 bp, Artificial Sequence
  caninized mouse antibody
atggccgtgctggggctgctcttctgcctggtgacattcccaagctgtgtgctaagcgaggtgcagctggtgcagtccggcggcgatctggtgaagcctggaggcagcgtgagactgagctgcgtggccagcggctacaccttcaccagctactacctgtactgggtgaggcaggctcctggcaaaggactgcagtggatcggcggcgtgaatcctagcaacggcggcaccaacttcagcgagaagttcaagagcagggccaccctgagcgtggacaaggccaagaacaccgcctacatgcagctgaactccctgagggccgaggacaccgccgtgtactactgcaccaggagggacagcaactacgacggcggcttcgactactggggacagggaaccctgctgaccgtgtccagcgcttccacaacggctccgtcggtgtttcccctggcacctagctgcgggtcgacctcgggtagcacagtggcgctggcgtgtttggtgtcgggatactttcccgagccggtaacggtgtcatggaactcagggtcacttacatcaggagtccatacttttccgtccgtgctgcagtcaagcggcttgcattcactgtcctcgatggtgacggtgccttcgtcgaggtggcccagcgaaacgttcacttgtaacgtagtacacccggcctccaacacgaaagtcgataaaccggtattcaatgagtgcagatgtacagacacccctccctgtccggtacccgaaccccttggagggccgagcgtcctcatcttccctcccaagccaaaagacatcttgcgcattacgaggacaccagaagtcacgtgcgtagtgcttgatctcggtagagaagatcccgaggtccagatctcgtggtttgtggatggaaaggaggtccacaccgcaaagactcagtcgcgcgagcagcagttcaatggcacgtatcgggtcgtgagcgtgcttcctatcgagcatcaggactggctcaccgggaaggagttcaaatgccgggtcaatcatatcgacctcccgtcaccaatcgagcggaccatctcgaaggctagaggaagggcgcacaaaccttcggtctatgtgcttcccccatcgcccaaagagctttcctcgtcggatacggtgtccattacatgcttgattaaggacttctatcctcctgatattgatgtggaatggcaatcaaacggacagcaggagccggaacgcaagcaccgaatgaccccaccgcaattggacgaagatggtagctactttctctactcaaagctctcagtcgacaaatcccgatggcagcagggagatcccttcacttgcgccgtgatgcacgagacactccaaaatcattacacggacctttcgttgagccactcgcccggaaag

SEQ ID NO: 40 - protein, 470 aa, Artificial Sequence
  caninized mouse antibody
MAVLGLLFCLVTFPSCVLSEVQLVQSGGDLVKPGGSVRLSCVASGYTFTSYYLYWVRQAPGKGLQWIGGVNPSNGGTNFSEKFKSRATLSVDKAKNTAYMQLNSLRAEDTAVYYCTRRDSNYDGGFDYWGQGTLLTVSSASTTAPSVFPLAPSCGSTSGSTVALACLVSGYFPEPVTVSWNSGSLTSGVHTFPSVLQSSGLHSLSSMVTVPSSRWPSETFTCNVVHPASNTKVDKPVFNECRCTDTPPCPVPEPLGGPSVLIFPPKPKDILRITRTPEVTCVVLDLGREDPEVQISWFVDGKEVHTAKTQSREQQFNGTYRVVSVLPIEHQDWLTGKEFKCRVNHIDLPSPIERTISKARGRAHKPSVYVLPPSPKELSSSDTVSITCLIKDFYPPDIDVEWQSNGQQEPERKHRMTPPQLDEDGSYFLYSKLSVDKSRWQQGDPFTCAVMHETLQNHYTDLSLSHSPGK

SEQ ID NO: 41 - DNA, 1425 bp, Artificial Sequence
  caninized mouse antibody
atggccgtgctggggctgctcttctgcctggtgacattcccaagctgtgtgctaagcgaggtgcagctggtgcagtccggcggcgatctggtgaagcctggaggcagcgtgagactgagctgcgtggccagcggctacaccttcaccagctactacctgtactgggtgaggcaggctcctggcaaaggactgcagtggatcggcggcgtgaatcctagcaacggcggcaccaacttcagcgagaagttcaagagcagggccaccctgagcgtggacaaggccaagaacaccgcctacatgcagctgaactccctgagggccgaggacaccgccgtgtactactgcaccaggagggacagcaactacgacggcggcttcgactactggggacagggaaccctgctgaccgtgtccagcgcttccacaaccgcgccatcagtctttccgttggccccatcatgcgggtcgacgagcggatcgactgtggccctggcgtgcttggtgtcgggatactttcccgaacccgtcacggtcagctggaactccggatcgcttacgagcggtgtgcatacgttcccctcggtcttgcaatcatcagggctctactcgctgtcgagcatggtaacggtgccctcatcgaggtggccctccgaaacgttcacatgtaacgtagcacatccagcctccaaaaccaaggtggataaacccgtgccgaaaagagagaatgggcgggtgcctcgaccccctgattgccccaagtgtccggctccggaaatgctcggtggaccctcagtgtttatcttccctccgaagcccaaggacactctgctgatcgcgcgcactccagaagtaacatgtgtagtggtggaccttgatcccgaggaccccgaagtccagatctcctggtttgtagatgggaaacagatgcagaccgcaaaaactcaacccagagaggagcagttcaacggaacataccgagtggtatccgtccttccgattggccaccaggactggttgaaagggaagcagtttacgtgtaaagtcaacaataaggcgttgcctagccctattgagcggacgatttcgaaagctaggggacaggcccaccagccatcggtctatgtccttccgccttcccgcgaggagctctcgaagaatacagtgagccttacatgcctcattaaggatttcttcccgcctgatatcgacgtagagtggcaatcaaacggtcaacaggagccggaatccaagtatagaaccactccgccccagcttgacgaggacggatcatactttttgtattcaaaactgtcggtggataagagccggtggcagagaggtgacaccttcatctgtgcggtgatgcacgaagcactccataatcactacacccaagagagcctctcgcattcccccggaaagtga

SEQ ID NO: 42 - protein, 474 aa, Artificial Sequence
  caninized mouse antibody
MAVLGLLFCLVTFPSCVLSEVQLVQSGGDLVKPGGSVRLSCVASGYTFTSYYLYWVRQAPGKGLQWIGGVNPSNGGTNFSEKFKSRATLSVDKAKNTAYMQLNSLRAEDTAVYYCTRRDSNYDGGFDYWGQGTLLTVSSASTTAPSVFPLAPSCGSTSGSTVALACLVSGYFPEPVTVSWNSGSLTSGVHTFPSVLQSSGLYSLSSMVTVPSSRWPSETFTCNVAHPASKTKVDKPVPKRENGRVPRPPDCPKCPAPEMLGGPSVFIFPPKPKDTLLIARTPEVTCVVVDLDPEDPEVQISWFVDGKQMQTAKTQPREEQFNGTYRVVSVLPIGHQDWLKGKQFTCKVNNKALPSPIERTISKARGQAHQPSVYVLPPSREELSKNTVSLTCLIKDFFPPDIDVEWQSNGQQEPESKYRTTPPQLDEDGSYFLYSKLSVDKSRWQRGDTFICAVMHEALHNHYTQESLSHSPGK

SEQ ID NO: 43 - DNA, 1410 bp, Artificial Sequence
  caninized mouse antibody
atggccgtgctggggctgctcttctgcctggtgacattcccaagctgtgtgctaagcgaggtgcagctggtgcagtccggcggcgatctggtgaagcctggaggcagcgtgagactgagctgcgtggccagcggctacaccttcaccagctactacctgtactgggtgaggcaggctcctggcaaaggactgcagtggatcggcggcgtgaatcctagcaacggcggcaccaacttcagcgagaagttcaagagcagggccaccctgagcgtggacaaggccaagaacaccgcctacatgcagctgaactccctgagggccgaggacaccgccgtgtactactgcaccaggagggacagcaactacgacggcggcttcgactactggggacagggaaccctgctgaccgtgtccagcgcttcaaccacagcgccgagcgtgttccctctggcgccgtcgtgcggttccacctcgggatcaacagtggccctcgcctgtctcgtgagcggatactttccggagcctgtcacggtgtcgtggaatagcggatcactcacgtcgggcgtgcatacttttccatccgtcttgcaatcgagcggattgtactcactctcctcaaccgtcactgtcccctcgtcgcgctggccctcggagacttttacgtgcaatgtagtccatccggcgagcaacacgaaggtcgacaagcccgtacccaaggaatcaacatgcaagtgcatctcgccctgtcccgtccccgaatcccttggtggcccctcagtgtttatcttccctccgaagcctaaagacatcttgagaatcacaagaacaccggaaatcacgtgtgtggtccttgacttgggacgcgaggaccctgaggtacaaatctcgtggtttgtggacgggaaagaggtgcacacagcaaagacacaaccacgcgagcagcagtttaactcaacgtacagggtagtatccgtacttcccattgaacaccaggattggctcaccggtaaagaattcaaatgccgagtgaatcacatcgggcttcctagcccaattgagcggacgatttccaaagctaggggtcaggcccaccagccgagcgtatacgtgttgccgccctccccgaaggagctgtcatcgtcagatacggtaacgttgacgtgtctgatcaaagatttctttcctcccgaaattgatgtggaatggcaaagcaatgggcagcccgagcccgagtcaaagtaccatactactgcaccacagctggacgaagatggatcgtatttcctctactcgaaactgtccgtggataagtcccggtggcagcaaggggacaccttcacttgcgcggtcatgcacgaggcacttcagaaccactatacggacttgagcctctcgcattcgccagggaag

SEQ ID NO: 44 - protein, 470 aa, Artificial Sequence
  caninized mouse antibody
MAVLGLLFCLVTFPSCVLSEVQLVQSGGDLVKPGGSVRLSCVASGYTFTSYYLYWVRQAPGKGLQWIGGVNPSNGGTNFSEKFKSRATLSVDKAKNTAYMQLNSLRAEDTAVYYCTRRDSNYDGGFDYWGQGTLLTVSSASTTAPSVFPLAPSCGSTSGSTVALACLVSGYFPEPVTVSWNSGSLTSGVHTFPSVLQSSGLYSLSSTVTVPSSRWPSETFTCNVVHPASNTKVDKPVPKESTCKCISPCPVPESLGGPSVFIFPPKPKDILRITRTPEITCVVLDLGREDPEVQISWFVDGKEVHTAKTQPREQQFNSTYRVVSVLPIEHQDWLTGKEFKCRVNHIGLPSPIERTISKARGQAHQPSVYVLPPSPKELSSSDTVTLTCLIKDFFPPEIDVEWQSNGQPEPESKYHTTAPQLDEDGSYFLYSKLSVDKSRWQQGDTFTCAVMHEALQNHYTDLSLSHSPGK

SEQ ID NO: 45 - DNA, 732 bp, Artificial Sequence
  caninized mouse antibody
atggatatgagagtacctgcacaacttctgggattgctgcttctttggctgagaggggcccgctgcgatatcgtcctgacccagacccctctgagcctgtccgtgagccctggagaacccgccagcatcagctgcagggcctccaagagcgtgagcaccagcggcttcagctacctgcactggtacaggcagaagcccggacagagccctcagctgctgatcttcctggccagcaacctggagagcggcgtgcctgacaggtttagcggaagcggcagcggcaccgacttcacactgaggatctccagggtggaagccgacgacgccggagtgtactactgccagcacagctgggaactgcccctgaccttcggccagggcaccaaggtggagatcaagaggaacgacgctcagccagccgtgtacctcttccagccttcgccggaccagcttcatacggggtcagcgtcggtggtgtgcctgttgaactcgttttaccccaaggacattaacgtgaagtggaaggtagacggggtaattcaagacactggcattcaagagtccgtcacggaacaagactcaaaagactcaacgtattcactgtcgtcaaccttgacgatgtcaagcaccgagtatcttagccatgagctgtattcgtgcgagatcacccacaagtccctcccctccactcttatcaaatcctttcagcggtcggaatgtcagcgggtcgat

SEQ ID NO: 46 - protein, 244 aa, Artificial Sequence
  caninized mouse antibody
MDMRVPAQLLGLLLLWLRGARCDIVLTQTPLSLSVSPGEPASISCRASKSVSTSGFSYLHWYRQKPGQSPQLLIFLASNLESGVPDRFSGSGSGTDFTLRISRVEADDAGVYYCQHSWELPLTFGQGTKVEIKRNDAQPAVYLFQPSPDQLHTGSASVVCLLNSFYPKDINVKWKVDGVIQDTGIQESVTEQDSKDSTYSLSSTLTMSSTEYLSHELYSCEITHKSLPSTLIKSFQRSECQRVD

SEQ ID NO: 47 - DNA, 732 bp, Artificial Sequence
  caninized mouse antibody
atggatatgagagtacctgcacaacttctgggattgctgcttctttggctgagaggggcccgctgcgatatcgtcctgacccagacccctcctagcctgtccgtgagccctggagaacccgccagcatcagctgcagggcctccaagagcgtgagcaccagcggcttcagctacctgcactggtacaggcagaagcccggacagcctcctcagctgctgatcttcctggccagcaacctggagagcggcgtgcctgacaggtttagcggaagcggcagcggcaccgacttcacactgaggatctccagggtggaagccgacgacgccggagtgtactactgccagcacagctgggaactgcccctgaccttcggccagggcaccaaggtggagatcaagaggaacgacgctcagccagccgtgtacctcttccagccttcgccggaccagcttcatacggggtcagcgtcggtggtgtgcctgttgaactcgttttaccccaaggacattaacgtgaagtggaaggtagacggggtaattcaagacactggcattcaagagtccgtcacggaacaagactcaaaagactcaacgtattcactgtcgtcaaccttgacgatgtcaagcaccgagtatcttagccatgagctgtattcgtgcgagatcacccacaagtccctcccctccactcttatcaaatcctttcagcggtcggaatgtcagcgggtcgat

SEQ ID NO: 48 - protein, 244 aa, Artificial Sequence
  caninized mouse antibody
MDMRVPAQLLGLLLLWLRGARCDIVLTQTPPSLSVSPGEPASISCRASKSVSTSGFSYLHWYRQKPGQPPQLLIFLASNLESGVPDRFSGSGSGTDFTLRISRVEADDAGVYYCQHSWELPLTFGQGTKVEIKRNDAQPAVYLFQPSPDQLHTGSASVVCLLNSFYPKDINVKWKVDGVIQDTGIQESVTEQDSKDSTYSLSSTLTMSSTEYLSHELYSCEITHKSLPSTLIKSFQRSECQRVD

SEQ ID NO: 49 - protein, 336 aa, Canis familiaris
SASTTAPSVFPLAPSCGSTSGSTVALACLVSGYFPEPVTVSWNSGSLTSGVHTFPSVLQSSGLYSLSSMVTVPSSRWPSETFTCNVAHPASKTKVDKPVPKRENGRVPRPPDCPKCPAPEMLGGPSVFIFPPKPKDTLLIARTPEVTCVVVDLDPEDPEVQISWFVDGKQMQTAKTQPREEQFNGTYRVVSVLPIGHQDWLKGKQFTCKVNNKALPSPIERTISKARGQAHQPSVYVLPPSREELSKNTVSLTCLIKDFFPPDIDVEWQSNGQQEPESKYRTTPPQLDEDGSYFLYSKLSVDKSRWQRGDTFICAVMHEALHNHYTQESLSHSPGK

SEQ ID NO: 50 - protein, 331 aa, Artificial Sequence
  modified canine sequence
SASTTAPSVFPLAPSCGSTSGSTVALACLVSGYFPEPVTVSWNSGSLTSGVHTFPSVLQSSGLYSLSSMVTVPSSRWPSETFTCNVAHPASKTKVDKPVFNECRCTDTPPCPAPEMLGGPSVFIFPPKPKATLLIARTPEVTCVVVDLDPEDPEVQISWFVDGKQMQTAKTQPREEQFAGTYRVVSVLPIGHQDWLKGKQFTCKVNNKALPSPIERTISKARGQAHQPSVYVLPPSREELSKNTVSLTCLIKDFFPPDIDVEWQSNGQQEPESKYRTTPPQLDEDGSYFLYSKLSVDKSRWQRGDTFICAVMHEALHNHYTQESLSHSPGK

SEQ ID NO: 51 - protein, 331 aa, Artificial Sequence
  modified canine sequence
SASTTAPSVFPLAPSCGSTSGSTVALACLVSGYFPEPVTVSWNSGSLTSGVHTFPSVLQSSGLYSLSSMVTVPSSRWPSETFTCNVAHPASKTKVDKPVPKESTCKCISPCPAPEMLGGPSVFIFPPKPKATLLIARTPEVTCVVVDLDPEDPEVQISWFVDGKQMQTAKTQPREEQFAGTYRVVSVLPIGHQDWLKGKQFTCKVNNKALPSPIERTISKARGQAHQPSVYVLPPSREELSKNTVSLTCLIKDFFPPDIDVEWQSNGQQEPESKYRTTPPQLDEDGSYFLYSKLSVDKSRWQRGDTFICAVMHEALHNHYTQESLSHSPGK

SEQ ID NO: 52 - protein, 336 aa, Artificial Sequence
  modified canine sequence
SASTTAPSVFPLAPSCGSTSGSTVALACLVSGYFPEPVTVSWNSGSLTSGVHTFPSVLQSSGLYSLSSMVTVPSSRWPSETFTCNVAHPASKTKVDKPVPKRENGRVPRPPDCPKCPAPEMLGGPSVFIFPPKPKATLLIARTPEVTCVVVDLDPEDPEVQISWFVDGKQMQTAKTQPREEQFAGTYRVVSVLPIGHQDWLKGKQFTCKVNNKALPSPIERTISKARGQAHQPSVYVLPPSREELSKNTVSLTCLIKDFFPPDIDVEWQSNGQQEPESKYRTTPPQLDEDGSYFLYSKLSVDKSRWQRGDTFICAVMHEALHNHYTQESLSHSPGK

SEQ ID NO: 53 - protein, 401 aa, Artificial Sequence
  canine and human
MNFLLSWVHWSLALLLYLHHAKWSQALDSPDRPWSPLTFSPAQLTVQEGENATFTCSLADIPDSFVLNWYRLSPRNQTDKLAAFQEDRIEPGRDRRFRVMRLPNGRDFHMSIVAARLNDSGIYLCGAIYLPPNTQINESPRAELSVTERTLEPPTQSPSPPPRLSGQLQGLVGTDKTHTCPPCPAPELLGGPSVFLFPPKPKDTLMISRTPEVTCVVVDVSHEDPEVKFNWYVDGVEVHNAKTKPREEQYNSTYRVVSVLTVLHQDWLNGKEYKCKVSNKALPAPIEKTISKAKGQPREPQVYTLPPSRDELTKNQVSLTCLVKGFYPSDIAVEWESNGQPENNYKTTPPVLDSDGSFFLYSKLTVDKSRWQQGNVFSCSVMHEALHNHYTQKSLSLSPGK